European Patent Application EP 4 431 519 A1, published September 18, 2024. Title: Method for Producing Compound, Method for Producing Compound Library, Compound Library and Screening Method. Applicant: The University of Tokyo. The sequence listing filed with the application follows.

SEQUENCE LISTING (204 sequences)

SEQ ID NO: 1 - protein, 302 aa, Limnothrix sp. CACIAM 69d
MKKRKSSKVFKSTIAPEEKLRYIGNHKQAFDIEPLYPLALFEEFVATTGDCIIECSGKIKQDQLYPARIDLQFSDKHHFHNIHTSIDFLKRAASRTDVNLNLDILATFLAGNFDYSKVQNILAGIDLRQNLGESKLKLFIRIGDYPAKMAVAKHLCNITPESEAMLRSDTLHIGFDFYLDGRSAIELYPELKKDEFNHPFIYNQLKTILSPEALKPLPLCNLFGIGLSPANEANVLYYHLENIEDFLSYFPINDTARRVHDFYLQQEGSRRMWVALSESEMKAGRINNVNLYYSKAFTSQNP

SEQ ID NO: 2 - protein, 286 aa, Symploca sp. SIO1B1
MNQSRDKLLYIGRHKSAFDIDYLYPMDIFEQFVESTGDGLIECSGKIKQDKLYPARFDLQFSDRQYAKNIYASIDFLKRVATRVDVSLDLNLLEQFLGNDFDFSKVQTVLVGVDLRHELHESRLKLFIRIGDYPEKVTLAKKLCGDSPQLQQLLRYDTLHIGFDFNLDGRSAIELYPEVKKEEFKQPEVYQKLTEILSLAALKPLAISNLMGIGFSQANEAKVLYYHLENIRDFLNYFPINNVARRVHDFYLQQDGSKKMWVALSEAELIAGKINNVNLYYSKAFF

SEQ ID NO: 3 - protein, 289 aa, Dolichospermum circinale
MTTLLESGKKIYYIGIHKQIFEIKNFYPLDIFDSFVNQIETTSENCSLESSCKIELDKLYPARFGIGFTLKNLKQLNVVYEFFQKVESRIDVQINYSLIQQFFGENFDFNKMTEFMVGIDARQELSETKLKIALTIKNYPEKIKTAIALNGGLDKNIYNLLVSNSLHIGFDLSLDGRSEIELYPYIRNQEFQIFDIQQRLATVLSPQALQFLPICSRICVGLSKANADKVVYFYLKNLNDFLNYFTVNDTARRVHAYYQQQPMREMCVAVQEKQLLGGTIEKMNLYYLI

SEQ ID NO: 4 - protein, 290 aa, Dolichospermum sp. UKL201
MTTLLLQRGKEIYYIGIHKQIFEIKNFYPLDIFDSFVTQIETTSENCYLESSCKIERDKLYPARFGIGFTLKNLKQLNVVYEFFQKVESRIDVQINYSLIQQFFGEDFDFNKMTEFMVGVDARPELAESKLKIALTIKDYPEKIKTAIELNGGLDKNIYNLLVSNSLHIGFDLSLDGRSEIELYPYIRNQEFQIFDIQQRLATVLLPQSLQFLPICSRICVGLSKANADKVVYFYLKNLNDFLNYFTVNDTARRVHAYYQQQPMREMCVAVQEKQLLGGTIEKMNLYYLI

SEQ ID NO: 5 - protein, 288 aa, Microcystis aeruginosa
MKSNKKLYYISAHKHAFEIDNLYPLNLFEGFVERIEKIEKTENCVLESSCKIDHDKLYPVRFNIGFPNNSIKQLHAVMDFFRRVESRVDVKLNLSLFQQFIGNDFKLDKMTDLMLGIDLRRDLSDSRLKIGLTIEDYPEKQKAAVILNNNIDEVTSNLLISNRLHIGFDFYLNGRSEMELYPHIMQQDFQKLDVQQRLSKVLSPPALQVVPACTRICVGISKANRDKIIYYYLENMGDFLNYFTVNDTARKVHAYYLKQPVVEMCVALPESELLAGTTIKNLNLYYLL

SEQ ID NO: 6 - protein, 289 aa, Microcystis aeruginosa
MLKSNKKLYYISAHKHAFEIDNLYPLNLFEGFVERIEKIEKTENCVLESSCKIDHDKLYPVRFNIGFPNNSIKQLHAVMDFFRRVESRVDVKLNLSLFQQFIGNDFKLDKMTDLMLGIDLRRDLSDSRLKIGLTIEDYPEKQKAAVILNNNIDEVTSNLLISNRLHIGFDFYLNGRSEMELYPHIMQQDFQKLDVQQRLSKVLSPPALQVVPACTRICVGISKANRDKIIYYYLENMGDFLNYFTVNDTARKVHAYYLKQPVVEMCVALPESELLAGTTIKNLNLYYLL

SEQ ID NO: 7 - protein, 289 aa, Aphanizomenon sp. UHCC 0183
MTTLLQRGKEIYYIGIHKQIFEIKNFYPLDIFDSFVTQIETTSENCYLESSCKIERDKLYPARFGIGFTLKNLKQLNVVYEFFQKVESRIDVQINYSLIQQFFGEDFDFNKMTEFMVGVDARPELAESKLKIALTIKDYPEKIKTAIELNGGLDKNIYNLLVSNSLHIGFDLSLDGRSEIELYPYIRNQEFQIFDIQQRLATVLLPQSLQFLPICSRICVGLSKANADKVVYFYLKNLNDFLNYFTVNDTARRVHAYYQQQPMDEMCVAVQEKELLGGTIEKMNLYYLI

SEQ ID NO: 8 - protein, 287 aa, Dolichospermum sp. JUN01
MTTLLLQRGKEIYYIGIHKQIFEIKNFYPLDIFDSFVTQIETTSENCYLESSCKIERDKLYPARFGIGFTLKNLKQLNVVYEFFQKVESRIDVQINYSLIQQFFGEDFDFNKMTEFMVGVDARPELAESKLKIALTIKDYPEKIKTAIELNGGLDKNIYNLLVSNSLHIGFDLSLDGRSEIELYPYIRNQEFQIFDIQQRLATVLLPQSLPICSRICVGLSKANADKVVYFYLKNLNDFLNYFTVNDTARRVHAYYQQQPMREMCVAVQEKQLLGGTIEKMNLYYLI

SEQ ID NO: 9 - protein, 254 aa, Aphanizomenon flos-aquae FACHB-1040
MFRIKELQFYIYLESSCKIERDKLYPARFSIGFTLKNLKQLNVVYEFFQKVESRIDVQINYSLIQQFFGEDFDFNKMTEFMVGVDARPELAESKLKIALTIKDYPEKIKTAIELNGGLDKNIYNLLVSNSLHIGFDLSLDGRSEIELYPYIRNQEFQIFDIQQRLATVLLPQSLQFLPICSRICVGLSKANADKVVYFYLKNLNDFLNYFTVNDTARRVHAYYQQQPMDEMCVAVQEKELLGGTIEKMNLYYLI

SEQ ID NO: 10 - protein, 289 aa, Microcystis aeruginosa
MATSLESSKKNYYISTHKQAFDVENFYPLEIWEKFVEKIEKTSEKCFLESSCKIDQGQFYAARFGIGFDLQNLQQLNAVYNFCQEVESRVGVRVDYSLIKQFLGDDFDFSKMTEFLIGVDARRELAESKLKIALTINDYPEKLKTAIYLNGGLDETIEKLIVSNSLHLGFDLSLNGISEIELYPYIGKQDFQRIDIQQRLATVLSPQALRPLAACRRICVGLSKGNTEKILYYYLEDIKDFLNYFTPNDTARRVHAYYQKQPISEMCVAAPESQFIAEKIEKMNLYYLF

SEQ ID NO: 11 - protein, 187 aa, Dolichospermum sp. OL01
MTKKNIRPQQVAPVERETTSTAKDQSGQVTAQWCIDYPKKIKTAIELNGGLDKNIYNLLVSNSLHIGFDLSLDGRSEIELYPYIRNQEFQIFDIQQRLATVLLPQSLQFLPICSRICVGLSKANADKVVYFYLKNLNDFLNYFTVNDTARRVHAYYQQQPMREMCVAVQEKQLLGGTIEKMNLYYLI

SEQ ID NO: 12 - protein, 290 aa, Microcystis aeruginosa NIES-88
MVLKSNKKLYYISAHKHAFEIDNLYPLNLFEGFVERIEKIEKTENCVLESSCKIDHDKLYPVRFNIGFPNNSIKQLHAVMDFFRRVESRVDVKLNLSLFQQFIGNDFKLDKMTDLMLGIDLRRDLSDSRLKIGLTIEDYPEKQKAAVILNNNIDEVTSNLLISNRLHIGFDFYLNGRSEMELYPHIMQQDFQKLDVQQRLSKVLSPPALQVVPACTRICVGISKANRDKIIYYYLENMGDFLNYFTVNDTARKVHAYYLKQPVVEMCVALPESELLAGTTIKNLNLYYLL

SEQ ID NO: 13 - protein, 302 aa, synthetic construct
  REGION 1..302: note = LimF-H172L
MKKRKSSKVFKSTIAPEEKLRYIGNHKQAFDIEPLYPLALFEEFVATTGDCIIECSGKIKQDQLYPARIDLQFSDKHHFHNIHTSIDFLKRAASRTDVNLNLDILATFLAGNFDYSKVQNILAGIDLRQNLGESKLKLFIRIGDYPAKMAVAKHLCNITPESEAMLRSDTLLIGFDFYLDGRSAIELYPELKKDEFNHPFIYNQLKTILSPEALKPLPLCNLFGIGLSPANEANVLYYHLENIEDFLSYFPINDTARRVHDFYLQQEGSRRMWVALSESEMKAGRINNVNLYYSKAFTSQNP

SEQ ID NO: 14 - DNA, 22 bp, synthetic construct
  misc_feature 1..22: note = T7pcrF22
  source 1..22: mol_type = other DNA
ggcgtaatacgactcactatag

SEQ ID NO: 15 - DNA, 43 bp, synthetic construct
  misc_feature 1..43: note = T7exF43
  source 1..43: mol_type = other DNA
taatacgactcactatagggttaactttaacaaggagaaaaac

SEQ ID NO: 16 - DNA, 49 bp, synthetic construct
  misc_feature 1..49: note = teLimE2(P-1A)-R1
  source 1..49: mol_type = other DNA
acacggaatttcttcatgtgcataacgcatgtttttctccttgttaaag

SEQ ID NO: 17 - DNA, 49 bp, synthetic construct
  misc_feature 1..49: note = teLimE2(P-1D)-R1
  source 1..49: mol_type = other DNA
acacggaatttcttcatggtcataacgcatgtttttctccttgttaaag

SEQ ID NO: 18 - DNA, 49 bp, synthetic construct
  misc_feature 1..49: note = teLimE2(P-1E)-R1
  source 1..49: mol_type = other DNA
acacggaatttcttcatgttcataacgcatgtttttctccttgttaaag

SEQ ID NO: 19 - DNA, 49 bp, synthetic construct
  misc_feature 1..49: note = teLimE2(P-1F)-R1
  source 1..49: mol_type = other DNA
acacggaatttcttcatgaaaataacgcatgtttttctccttgttaaag

SEQ ID NO: 20 - DNA, 49 bp, synthetic construct
  misc_feature 1..49: note = teLimE2(P-1G)-R1
  source 1..49: mol_type = other DNA
acacggaatttcttcatgaccataacgcatgtttttctccttgttaaag

SEQ ID NO: 21 - DNA, 49 bp, synthetic construct
  misc_feature 1..49: note = teLimE2(P-1H)-R1
  source 1..49: mol_type = other DNA
acacggaatttcttcatgatgataacgcatgtttttctccttgttaaag

SEQ ID NO: 22 - DNA, 49 bp, synthetic construct
  misc_feature 1..49: note = teLimE2(P-1I)-R1
  source 1..49: mol_type = other DNA
acacggaatttcttcatgaatataacgcatgtttttctccttgttaaag

SEQ ID NO: 23 - DNA, 49 bp, synthetic construct
  misc_feature 1..49: note = teLimE2(P-1K)-R1
  source 1..49: mol_type = other DNA
acacggaatttcttcatgcttataacgcatgtttttctccttgttaaag

SEQ ID NO: 24 - DNA, 49 bp, synthetic construct
  misc_feature 1..49: note = teLimE2(P-1L)-R1
  source 1..49: mol_type = other DNA
acacggaatttcttcatgcagataacgcatgtttttctccttgttaaag

SEQ ID NO: 25 - DNA, 49 bp, synthetic construct
  misc_feature 1..49: note = teLimE2(P-1M)-R1
  source 1..49: mol_type = other DNA
acacggaatttcttcatgcatataacgcatgtttttctccttgttaaag

SEQ ID NO: 26 - DNA, 49 bp, synthetic construct
  misc_feature 1..49: note = teLimE2(P-1N)-R1
  source 1..49: mol_type = other DNA
acacggaatttcttcatgattataacgcatgtttttctccttgttaaag

SEQ ID NO: 27 - DNA, 49 bp, synthetic construct
  misc_feature 1..49: note = teLimE2-R1
  source 1..49: mol_type = other DNA
acacggaatttcttcatgcggataacgcatgtttttctccttgttaaag

SEQ ID NO: 28 - DNA, 49 bp, synthetic construct
  misc_feature 1..49: note = teLimE2(P-1Q)-R1
  source 1..49: mol_type = other DNA
acacggaatttcttcatgttgataacgcatgtttttctccttgttaaag

SEQ ID NO: 29 - DNA, 49 bp, synthetic construct
  misc_feature 1..49: note = teLimE2(P-1R)-R1
  source 1..49: mol_type = other DNA
acacggaatttcttcatgacgataacgcatgtttttctccttgttaaag

SEQ ID NO: 30 - DNA, 49 bp, synthetic construct
  misc_feature 1..49: note = teLimE2(P-1S)-R1
  source 1..49: mol_type = other DNA
acacggaatttcttcatgagaataacgcatgtttttctccttgttaaag

SEQ ID NO: 31 - DNA, 49 bp, synthetic construct
  misc_feature 1..49: note = teLimE2(P-1T)-R1
  source 1..49: mol_type = other DNA
acacggaatttcttcatgggtataacgcatgtttttctccttgttaaag

SEQ ID NO: 32 - DNA, 49 bp, synthetic construct
  misc_feature 1..49: note = teLimE2(P-1V)-R1
  source 1..49: mol_type = other DNA
acacggaatttcttcatgaacataacgcatgtttttctccttgttaaag

SEQ ID NO: 33 - DNA, 49 bp, synthetic construct
  misc_feature 1..49: note = teLimE2(P-1W)-R1
  source 1..49: mol_type = other DNA
acacggaatttcttcatggcaataacgcatgtttttctccttgttaaag

SEQ ID NO: 34 - DNA, 49 bp, synthetic construct
  misc_feature 1..49: note = teLimE2(P-1Y)-R1
  source 1..49: mol_type = other DNA
acacggaatttcttcatgataataacgcatgtttttctccttgttaaag

SEQ ID NO: 35 - DNA, 27 bp, synthetic construct
  misc_feature 1..27: note = teLimE2-R2
  source 1..27: mol_type = other DNA
cgaagcttaacacggaatttcttcatg

SEQ ID NO: 36 - DNA, 37 bp, synthetic construct
  misc_feature 1..37: note = teLimE2(E+1A)-R1
  source 1..37: mol_type = other DNA
tgcatgcggataacgcatgtttttctccttgttaaag

SEQ ID NO: 37 - DNA, 37 bp, synthetic construct
  misc_feature 1..37: note = teLimE2(E+1D)-R1
  source 1..37: mol_type = other DNA
gtcatgcggataacgcatgtttttctccttgttaaag

SEQ ID NO: 38 - DNA, 37 bp, synthetic construct
  misc_feature 1..37: note = teLimE2(E+1F)-R1
  source 1..37: mol_type = other DNA
aaaatgcggataacgcatgtttttctccttgttaaag

SEQ ID NO: 39 - DNA, 37 bp, synthetic construct
  misc_feature 1..37: note = teLimE2(E+1G)-R1
  source 1..37: mol_type = other DNA
accatgcggataacgcatgtttttctccttgttaaag

SEQ ID NO: 40 - DNA, 37 bp, synthetic construct
  misc_feature 1..37: note = teLimE2(E+1H)-R1
  source 1..37: mol_type = other DNA
atgatgcggataacgcatgtttttctccttgttaaag

SEQ ID NO: 41 - DNA, 37 bp, synthetic construct
  misc_feature 1..37: note = teLimE2(E+1I)-R1
  source 1..37: mol_type = other DNA
aatatgcggataacgcatgtttttctccttgttaaag

SEQ ID NO: 42 - DNA, 37 bp, synthetic construct
  misc_feature 1..37: note = teLimE2(E+1K)-R1
  source 1..37: mol_type = other DNA
cttatgcggataacgcatgtttttctccttgttaaag

SEQ ID NO: 43 - DNA, 37 bp, synthetic construct
  misc_feature 1..37: note = teLimE2(E+1L)-R1
  source 1..37: mol_type = other DNA
cagatgcggataacgcatgtttttctccttgttaaag

SEQ ID NO: 44 - DNA, 37 bp, synthetic construct
  misc_feature 1..37: note = teLimE2(E+1M)-R1
  source 1..37: mol_type = other DNA
catatgcggataacgcatgtttttctccttgttaaag

SEQ ID NO: 45 - DNA, 37 bp, synthetic construct
  misc_feature 1..37: note = teLimE2(E+1N)-R1
  source 1..37: mol_type = other DNA
attatgcggataacgcatgtttttctccttgttaaag

SEQ ID NO: 46 - DNA, 37 bp, synthetic construct
  misc_feature 1..37: note = teLimE2(E+1P)-R1
  source 1..37: mol_type = other DNA
cggatgcggataacgcatgtttttctccttgttaaag

SEQ ID NO: 47 - DNA, 37 bp, synthetic construct
  misc_feature 1..37: note = teLimE2(E+1Q)-R1
  source 1..37: mol_type = other DNA
ttgatgcggataacgcatgtttttctccttgttaaag

SEQ ID NO: 48 - DNA, 37 bp, synthetic construct
  misc_feature 1..37: note = teLimE2(E+1R)-R1
  source 1..37: mol_type = other DNA
acgatgcggataacgcatgtttttctccttgttaaag

SEQ ID NO: 49 - DNA, 37 bp, synthetic construct
  misc_feature 1..37: note = teLimE2(E+1S)-R1
  source 1..37: mol_type = other DNA
agaatgcggataacgcatgtttttctccttgttaaag

SEQ ID NO: 50 - DNA, 37 bp, synthetic construct
  misc_feature 1..37: note = teLimE2(E+1T)-R1
  source 1..37: mol_type = other DNA
ggtatgcggataacgcatgtttttctccttgttaaag

SEQ ID NO: 51 - DNA, 37 bp, synthetic construct
  misc_feature 1..37: note = teLimE2(E+1V)-R1
  source 1..37: mol_type = other DNA
aacatgcggataacgcatgtttttctccttgttaaag

SEQ ID NO: 52 - DNA, 37 bp, synthetic construct
  misc_feature 1..37: note = teLimE2(E+1W)-R1
  source 1..37: mol_type = other DNA
gcaatgcggataacgcatgtttttctccttgttaaag

SEQ ID NO: 53 - DNA, 37 bp, synthetic construct
  misc_feature 1..37: note = teLimE2(E+1Y)-R1
  source 1..37: mol_type = other DNA
ataatgcggataacgcatgtttttctccttgttaaag

SEQ ID NO: 54 - DNA, 40 bp, synthetic construct
  misc_feature 1..40: note = teLimE2(E+1A)-R2
  source 1..40: mol_type = other DNA
cgaagcttaacacggaatttctgcatgcggataacgcatg

SEQ ID NO: 55 - DNA, 40 bp, synthetic construct
  misc_feature 1..40: note = teLimE2(E+1D)-R2
  source 1..40: mol_type = other DNA
cgaagcttaacacggaatttcgtcatgcggataacgcatg

SEQ ID NO: 56 - DNA, 40 bp, synthetic construct
  misc_feature 1..40: note = teLimE2(E+1F)-R2
  source 1..40: mol_type = other DNA
cgaagcttaacacggaatttcaaaatgcggataacgcatg

SEQ ID NO: 57 - DNA, 40 bp, synthetic construct
  misc_feature 1..40: note = teLimE2(E+1G)-R2
  source 1..40: mol_type = other DNA
cgaagcttaacacggaatttcaccatgcggataacgcatg

SEQ ID NO: 58 - DNA, 40 bp, synthetic construct
  misc_feature 1..40: note = teLimE2(E+1H)-R2
  source 1..40: mol_type = other DNA
cgaagcttaacacggaatttcatgatgcggataacgcatg

SEQ ID NO: 59 - DNA, 40 bp, synthetic construct
  misc_feature 1..40: note = teLimE2(E+1I)-R2
  source 1..40: mol_type = other DNA
cgaagcttaacacggaatttcaatatgcggataacgcatg

SEQ ID NO: 60 - DNA, 40 bp, synthetic construct
  misc_feature 1..40: note = teLimE2(E+1K)-R2
  source 1..40: mol_type = other DNA
cgaagcttaacacggaatttccttatgcggataacgcatg

SEQ ID NO: 61 - DNA, 40 bp, synthetic construct
  misc_feature 1..40: note = teLimE2(E+1L)-R2
  source 1..40: mol_type = other DNA
cgaagcttaacacggaatttccagatgcggataacgcatg

SEQ ID NO: 62 - DNA, 40 bp, synthetic construct
  misc_feature 1..40: note = teLimE2(E+1M)-R2
  source 1..40: mol_type = other DNA
cgaagcttaacacggaatttccatatgcggataacgcatg

SEQ ID NO: 63 - DNA, 40 bp, synthetic construct
  misc_feature 1..40: note = teLimE2(E+1N)-R2
  source 1..40: mol_type = other DNA
cgaagcttaacacggaatttcattatgcggataacgcatg

SEQ ID NO: 64 - DNA, 40 bp, synthetic construct
  misc_feature 1..40: note = teLimE2(E+1P)-R2
  source 1..40: mol_type = other DNA
cgaagcttaacacggaatttccggatgcggataacgcatg

SEQ ID NO: 65 - DNA, 40 bp, synthetic construct
  misc_feature 1..40: note = teLimE2(E+1Q)-R2
  source 1..40: mol_type = other DNA
cgaagcttaacacggaatttcttgatgcggataacgcatg

SEQ ID NO: 66 - DNA, 40 bp, synthetic construct
  misc_feature 1..40: note = teLimE2(E+1R)-R2
  source 1..40: mol_type = other DNA
cgaagcttaacacggaatttcacgatgcggataacgcatg

SEQ ID NO: 67 - DNA, 40 bp, synthetic construct
  misc_feature 1..40: note = teLimE2(E+1S)-R2
  source 1..40: mol_type = other DNA
cgaagcttaacacggaatttcagaatgcggataacgcatg

SEQ ID NO: 68 - DNA, 40 bp, synthetic construct
  misc_feature 1..40: note = teLimE2(E+1T)-R2
  source 1..40: mol_type = other DNA
cgaagcttaacacggaatttcggtatgcggataacgcatg

SEQ ID NO: 69 - DNA, 40 bp, synthetic construct
  misc_feature 1..40: note = teLimE2(E+1V)-R2
  source 1..40: mol_type = other DNA
cgaagcttaacacggaatttcaacatgcggataacgcatg

SEQ ID NO: 70 - DNA, 40 bp, synthetic construct
  misc_feature 1..40: note = teLimE2(E+1W)-R2
  source 1..40: mol_type = other DNA
cgaagcttaacacggaatttcgcaatgcggataacgcatg

SEQ ID NO: 71 - DNA, 40 bp, synthetic construct
  misc_feature 1..40: note = teLimE2(E+1Y)-R2
  source 1..40: mol_type = other DNA
cgaagcttaacacggaatttcataatgcggataacgcatg

SEQ ID NO: 72 - DNA, 59 bp, synthetic construct
  misc_feature 1..59: note = teMP(18aa)-R1
  source 1..59: mol_type = other DNA
ccggaatttctgcatgagaatatgcttgaccaacacgcatgtttttctccttgttaaag

SEQ ID NO: 73 - DNA, 56 bp, synthetic construct
  misc_feature 1..56: note = teMP(16aa)-R1
  source 1..56: mol_type = other DNA
ccggaatttctgcatgagaatatgcttgaacacgcatgtttttctccttgttaaag

SEQ ID NO: 74 - DNA, 44 bp, synthetic construct
  misc_feature 1..44: note = teMP(14aa)-R1
  source 1..44: mol_type = other DNA
ctgcatgagaatatgcttgacgcatgtttttctccttgttaaag

SEQ ID NO: 75 - DNA, 44 bp, synthetic construct; identical to SEQ ID NO: 74
  misc_feature 1..44: note = teMP(13aa)-R1
  source 1..44: mol_type = other DNA

SEQ ID NO: 76 - DNA, 44 bp, synthetic construct
  misc_feature 1..44: note = teMP(12aa)-R1
  source 1..44: mol_type = other DNA
tttctgcatgagaatatgcacgcatgtttttctccttgttaaag

SEQ ID NO: 77 - DNA, 44 bp, synthetic construct; identical to SEQ ID NO: 76
  misc_feature 1..44: note = teMP(11aa)-R1
  source 1..44: mol_type = other DNA

SEQ ID NO: 78 - DNA, 44 bp, synthetic construct
  misc_feature 1..44: note = teMP(10aa)-R1
  source 1..44: mol_type = other DNA
gaatttctgcatgagaataacgcatgtttttctccttgttaaag

SEQ ID NO: 79 - DNA, 41 bp, synthetic construct
  misc_feature 1..41: note = teMP(9aa)-R1
  source 1..41: mol_type = other DNA
gaatttctgcatgagaacgcatgtttttctccttgttaaag

SEQ ID NO: 80 - DNA, 40 bp, synthetic construct
  misc_feature 1..40: note = teMP(8aa)-R1
  source 1..40: mol_type = other DNA
aatttctgcatgagaacgcatgtttttctccttgttaaag

SEQ ID NO: 81 - DNA, 40 bp, synthetic construct
  misc_feature 1..40: note = teMP(7aa)-R1
  source 1..40: mol_type = other DNA
acattctgcatgagaacgcatgtttttctccttgttaaag

SEQ ID NO: 82 - DNA, 40 bp, synthetic construct
  misc_feature 1..40: note = teMP(6aa)-R1
  source 1..40: mol_type = other DNA
ttaacatgcatgagaacgcatgtttttctccttgttaaag

SEQ ID NO: 83 - DNA, 43 bp, synthetic construct
  misc_feature 1..43: note = teMP(5aa)-R1
  source 1..43: mol_type = other DNA
cgaagcttaacatgcatgagacatgtttttctccttgttaaag

SEQ ID NO: 84 - DNA, 40 bp, synthetic construct
  misc_feature 1..40: note = teMP(4aa)-R1
  source 1..40: mol_type = other DNA
cgaagcttaacaatgagacatgtttttctccttgttaaag

SEQ ID NO: 85 - DNA, 37 bp, synthetic construct
  misc_feature 1..37: note = teMP(3aa)-R1
  source 1..37: mol_type = other DNA
cgaagcttaacaatgcatgtttttctccttgttaaag

SEQ ID NO: 86 - DNA, 44 bp, synthetic construct
  misc_feature 1..44: note = teMP(18aa)-R2
  source 1..44: mol_type = other DNA
cgaagcttaacaacgttctgcttccggaatttctgcatgagaat

SEQ ID NO: 87 - DNA, 44 bp, synthetic construct
  misc_feature 1..44: note = teMP(16aa)-R2
  source 1..44: mol_type = other DNA
cgaagcttaacaacgtgcttccggaatttctgcatgagaatatg

SEQ ID NO: 88 - DNA, 44 bp, synthetic construct
  misc_feature 1..44: note = teMP(14aa)-R2
  source 1..44: mol_type = other DNA
cgaagcttaacatgcttccggaatttctgcatgagaatatgctt

SEQ ID NO: 89 - DNA, 44 bp, synthetic construct
  misc_feature 1..44: note = teMP(13aa)-R2
  source 1..44: mol_type = other DNA
cgaagcttaacatgccggaatttctgcatgagaatatgcttgac

SEQ ID NO: 90 - DNA, 41 bp, synthetic construct
  misc_feature 1..41: note = teMP(12aa)-R2
  source 1..41: mol_type = other DNA
cgaagcttaacatgccggaatttctgcatgagaatatgcac

SEQ ID NO: 91 - DNA, 38 bp, synthetic construct
  misc_feature 1..38: note = teMP(11aa)-R2
  source 1..38: mol_type = other DNA
cgaagcttaacacggaatttctgcatgagaatatgcac

SEQ ID NO: 92 - DNA, 34 bp, synthetic construct
  misc_feature 1..34: note = teMP(10aa)-R2
  source 1..34: mol_type = other DNA
cgaagcttaacacggaatttctgcatgagaataa

SEQ ID NO: 93 - DNA, 34 bp, synthetic construct
  misc_feature 1..34: note = teMP(9aa)-R2
  source 1..34: mol_type = other DNA
cgaagcttaacacggaatttctgcatgagaacgc

SEQ ID NO: 94 - DNA, 33 bp, synthetic construct
  misc_feature 1..33: note = teMP(8aa)-R2
  source 1..33: mol_type = other DNA
cgaagcttaacaaatttctgcatgagaacgcat

SEQ ID NO: 95 - DNA, 32 bp, synthetic construct
  misc_feature 1..32: note = teMP(7aa)-R2
  source 1..32: mol_type = other DNA
cgaagcttaacattctgcatgagaacgcatgt

SEQ ID NO: 96 - DNA, 27 bp, synthetic construct
  misc_feature 1..27: note = teMP(6aa)-R2
  source 1..27: mol_type = other DNA
cgaagcttaacatgcatgagaacgcat

SEQ ID NO: 97 - DNA, 18 bp, synthetic construct
  misc_feature 1..18: note = teMP(5aa)-R2
  source 1..18: mol_type = other DNA
cgaagcttaacatgcatg

SEQ ID NO: 98 - DNA, 18 bp, synthetic construct
  misc_feature 1..18: note = teMP(4aa)-R2
  source 1..18: mol_type = other DNA
cgaagcttaacaatgaga

SEQ ID NO: 99 - DNA, 18 bp, synthetic construct
  misc_feature 1..18: note = teMP(3aa)-R2
  source 1..18: mol_type = other DNA
cgaagcttaacaatgcat

SEQ ID NO: 100 - DNA, 44 bp, synthetic construct
  misc_feature 1..44: note = teR1-R1
  source 1..44: mol_type = other DNA
attcatgcggataacgcggaatcatgtttttctccttgttaaag

SEQ ID NO: 101 - DNA, 44 bp, synthetic construct
  misc_feature 1..44: note = teR2-R1
  source 1..44: mol_type = other DNA
accaatgggtgtcaccattcagcatgtttttctccttgttaaag

SEQ ID NO: 102 - DNA, 43 bp, synthetic construct
  misc_feature 1..43: note = teR3-R1
  source 1..43: mol_type = other DNA
agaagcatcaaacaaagacatgtttttctccttgttaaagtta

SEQ ID NO: 103 - DNA, 49 bp, synthetic construct
  misc_feature 1..49: note = teR4-R1
  source 1..49: mol_type = other DNA
aaactgagacgaaccataaagcaaatacatgtttttctccttgttaaag

SEQ ID NO: 104 - DNA, 47 bp, synthetic construct
  misc_feature 1..47: note = teR5-R1
  source 1..47: mol_type = other DNA
acggatgcggcggaacaataagatacatgtttttctccttgttaaag

SEQ ID NO: 105 - DNA, 31 bp, synthetic construct
  misc_feature 1..31: note = teR1-R2
  source 1..31: mol_type = other DNA
cgaagcttaacattcatgcggataacgcgga

SEQ ID NO: 106 - DNA, 43 bp, synthetic construct
  misc_feature 1..43: note = teR2-R2
  source 1..43: mol_type = other DNA
cgaagcttaacaacccggaccagaccaatgggtgtcaccattc

SEQ ID NO: 107 - DNA, 52 bp, synthetic construct
  misc_feature 1..52: note = teR3-R2
  source 1..52: mol_type = other DNA
cgaagcttagcaactataattagcaatataatgttcagaagcatcaaacaaa

SEQ ID NO: 108 - DNA, 46 bp, synthetic construct
  misc_feature 1..46: note = teR4-R2
  source 1..46: mol_type = other DNA
cgaagcttagcactgcggaatatgccaaaactgagacgaaccataa

SEQ ID NO: 109 - DNA, 44 bp, synthetic construct
  misc_feature 1..44: note = teR5-R2
  source 1..44: mol_type = other DNA
cgaagcttagcactcccgaggatacggatgcggcggaacaataa

SEQ ID NO: 110 - DNA, 40 bp, synthetic construct
  misc_feature 1..40: note = teR1(P-1K)-R1
  source 1..40: mol_type = other DNA
atgcttataacgcggaatcatgtttttctccttgttaaag

SEQ ID NO: 111 - DNA, 44 bp, synthetic construct
  misc_feature 1..44: note = teR2(W+1P)-R1
  source 1..44: mol_type = other DNA
acggatgggtgtcaccattcagcatgtttttctccttgttaaag

SEQ ID NO: 112 - DNA, 47 bp, synthetic construct
  misc_feature 1..47: note = teR5(P+1A)-R1
  source 1..47: mol_type = other DNA
atgcatgcggcggaacaataagatacatgtttttctccttgttaaag

SEQ ID NO: 113 - DNA, 34 bp, synthetic construct
  misc_feature 1..34: note = teR1(P-1K)-R2
  source 1..34: mol_type = other DNA
cgaagcttaacattcatgcttataacgcggaatc

SEQ ID NO: 114 - DNA, 43 bp, synthetic construct
  misc_feature 1..43: note = teR2(W+1P)-R2
  source 1..43: mol_type = other DNA
cgaagcttaacaacccggaccagacggatgggtgtcaccattc

SEQ ID NO: 115 - DNA, 52 bp, synthetic construct
  misc_feature 1..52: note = teR3(E-1S)-R2
  source 1..52: mol_type = other DNA
cgaagcttagcaactataattagcaatataatgagaagaagcatcaaacaaa

SEQ ID NO: 116 - DNA, 47 bp, synthetic construct
  misc_feature 1..47: note = teR4(W-1A)-R2
  source 1..47: mol_type = other DNA
cgaagcttagcactgcggaatatgtgcaaactgagacgaaccataaa

SEQ ID NO: 117 - DNA, 44 bp, synthetic construct
  misc_feature 1..44: note = teR5(P+1A)-R2
  source 1..44: mol_type = other DNA
cgaagcttagcactcccgaggatatgcatgcggcggaacaataa

SEQ ID NO: 118 - DNA, 44 bp, synthetic construct
  misc_feature 1..44: note = teLimE2-CAC-R1
  source 1..44: mol_type = other DNA
gaatttcttcgtgcggataacgcatgtttttctccttgttaaag

SEQ ID NO: 119 - DNA, 32 bp, synthetic construct
  misc_feature 1..32: note = teLimE2-CAC-R2
  source 1..32: mol_type = other DNA
cgaagcttaacacggaatttcttcgtgcggat

SEQ ID NO: 120 - DNA, 56 bp, synthetic construct
  misc_feature 1..56: note = teR6-R1
  source 1..56: mol_type = other DNA
aagcttaacacggaatataggtatgattaccacgcatgtttttctccttgttaaag

SEQ ID NO: 121 - DNA, 44 bp, synthetic construct
  misc_feature 1..44: note = teR6-H5A-R1
  source 1..44: mol_type = other DNA
gaatataggttgcattaccacgcatgtttttctccttgttaaag

SEQ ID NO: 122 - DNA, 44 bp, synthetic construct
  misc_feature 1..44: note = teR6-H5A(T-1A)-R1
  source 1..44: mol_type = other DNA
gaatatatgctgcattaccacgcatgtttttctccttgttaaag

SEQ ID NO: 123 - DNA, 44 bp, synthetic construct
  misc_feature 1..44: note = teR6-H5A(T-1D)-R1
  source 1..44: mol_type = other DNA
gaatatagtctgcattaccacgcatgtttttctccttgttaaag

SEQ ID NO: 124 - DNA, 44 bp, synthetic construct
  misc_feature 1..44: note = teR6-H5A(T-1E)-R1
  source 1..44: mol_type = other DNA
gaatatattctgcattaccacgcatgtttttctccttgttaaag

SEQ ID NO: 125 - DNA, 44 bp, synthetic construct
  misc_feature 1..44: note = teR6-H5A(T-1F)-R1
  source 1..44: mol_type = other DNA
gaatataaaatgcattaccacgcatgtttttctccttgttaaag

SEQ ID NO: 126 - DNA, 44 bp, synthetic construct
  misc_feature 1..44: note = teR6-H5A(T-1G)-R1
  source 1..44: mol_type = other DNA
gaatataacctgcattaccacgcatgtttttctccttgttaaag

SEQ ID NO: 127 - DNA, 44 bp, synthetic construct
  misc_feature 1..44: note = teR6-H5A(T-1H)-R1
  source 1..44: mol_type = other DNA
gaatataatgtgcattaccacgcatgtttttctccttgttaaag

SEQ ID NO: 128 - DNA, 44 bp, synthetic construct
  misc_feature 1..44: note = teR6-H5A(T-1I)-R1
  source 1..44: mol_type = other DNA
gaatataaattgcattaccacgcatgtttttctccttgttaaag

SEQ ID NO: 129 - DNA, 44 bp, synthetic construct
  misc_feature 1..44: note = teR6-H5A(T-1K)-R1
  source 1..44: mol_type = other DNA
gaatatactttgcattaccacgcatgtttttctccttgttaaag

SEQ ID NO: 130 - DNA, 44 bp, synthetic construct
  misc_feature 1..44: note = teR6-H5A(T-1L)-R1
  source 1..44: mol_type = other DNA
gaatatacagtgcattaccacgcatgtttttctccttgttaaag

SEQ ID NO: 131 - DNA, 44 bp, synthetic construct
  misc_feature 1..44: note = teR6-H5A(T-1M)-R1
  source 1..44: mol_type = other DNA
gaatatacattgcattaccacgcatgtttttctccttgttaaag

SEQ ID NO: 132 - DNA, 44 bp, synthetic construct
  misc_feature 1..44: note = teR6-H5A(T-1N)-R1
  source 1..44: mol_type = other DNA
gaatataatttgcattaccacgcatgtttttctccttgttaaag

SEQ ID NO: 133 - DNA, 44 bp, synthetic construct
  misc_feature 1..44: note = teR6-H5A(T-1P)-R1
  source 1..44: mol_type = other DNA
gaatatacggtgcattaccacgcatgtttttctccttgttaaag

SEQ ID NO: 134 - DNA, 44 bp, synthetic construct
  misc_feature 1..44: note = teR6-H5A(T-1Q)-R1
  source 1..44: mol_type = other DNA
gaatatattgtgcattaccacgcatgtttttctccttgttaaag

SEQ ID NO: 135 - DNA, 44 bp, synthetic construct
  misc_feature 1..44: note = teR6-H5A(T-1R)-R1
  source 1..44: mol_type = other DNA
gaatataacgtgcattaccacgcatgtttttctccttgttaaag

SEQ ID NO: 136 - DNA, 44 bp, synthetic construct
  misc_feature 1..44: note = teR6-H5A(T-1S)-R1
  source 1..44: mol_type = other DNA
gaatataagatgcattaccacgcatgtttttctccttgttaaag

SEQ ID NO: 137 - DNA, 44 bp, synthetic construct
  misc_feature 1..44: note = teR6-H5A(T-1V)-R1
  source 1..44: mol_type = other DNA
gaatataaactgcattaccacgcatgtttttctccttgttaaag

SEQ ID NO: 138 - DNA, 44 bp, synthetic construct
  misc_feature 1..44: note = teR6-H5A(T-1W)-R1
  source 1..44: mol_type = other DNA
gaatataccatgcattaccacgcatgtttttctccttgttaaag

SEQ ID NO: 139 - DNA, 44 bp, synthetic construct
  misc_feature 1..44: note = teR6-H5A(T-1Y)-R1
  source 1..44: mol_type = other DNA
gaatataatatgcattaccacgcatgtttttctccttgttaaag

SEQ ID NO: 140 - DNA, 22 bp, synthetic construct
  misc_feature 1..22: note = teR6-R2
  source 1..22: mol_type = other DNA
cgaagcttaacacggaatatag

SEQ ID NO: 141 - DNA, 33 bp, synthetic construct
  misc_feature 1..33: note = teR6-H5A-R2
  source 1..33: mol_type = other DNA
cgaagcttaacacggaatataggttgcattacc

SEQ ID NO: 142 - DNA, 33 bp, synthetic construct
  misc_feature 1..33: note = teR6-H5A(T-1A)-R2
  source 1..33: mol_type = other DNA
cgaagcttaacacggaatatatgctgcattacc

SEQ ID NO: 143 - DNA, 33 bp, synthetic construct
  misc_feature 1..33: note = teR6-H5A(T-1D)-R2
  source 1..33: mol_type = other DNA
cgaagcttaacacggaatatagtctgcattacc

SEQ ID NO: 144 - DNA, 33 bp, synthetic construct
  misc_feature 1..33: note = teR6-H5A(T-1E)-R2
  source 1..33: mol_type = other DNA
cgaagcttaacacggaatatattctgcattacc

SEQ ID NO: 145 - DNA, 33 bp, synthetic construct
  misc_feature 1..33: note = teR6-H5A(T-1F)-R2
  source 1..33: mol_type = other DNA
cgaagcttaacacggaatataaaatgcattacc

SEQ ID NO: 146 - DNA, 33 bp, synthetic construct
  misc_feature 1..33: note = teR6-H5A(T-1G)-R2
  source 1..33: mol_type = other DNA
cgaagcttaacacggaatataacctgcattacc

SEQ ID NO: 147 - DNA, 33 bp, synthetic construct
  misc_feature 1..33: note = teR6-H5A(T-1H)-R2
  source 1..33: mol_type = other DNA
cgaagcttaacacggaatataatgtgcattacc

SEQ ID NO: 148 - DNA, 33 bp, synthetic construct
  misc_feature 1..33: note = teR6-H5A(T-1I)-R2
  source 1..33: mol_type = other DNA
cgaagcttaacacggaatataaattgcattacc

SEQ ID NO: 149 - DNA, 33 bp, synthetic construct
  misc_feature 1..33: note = teR6-H5A(T-1K)-R2
  source 1..33: mol_type = other DNA
cgaagcttaacacggaatatactttgcattacc

SEQ ID NO: 150 - DNA, 33 bp, synthetic construct
  misc_feature 1..33: note = teR6-H5A(T-1L)-R2
  source 1..33: mol_type = other DNA
cgaagcttaacacggaatatacagtgcattacc

SEQ ID NO: 151 - DNA, 33 bp, synthetic construct
  misc_feature 1..33: note = teR6-H5A(T-1M)-R2
  source 1..33: mol_type = other DNA
cgaagcttaacacggaatatacattgcattacc

SEQ ID NO: 152 - DNA, 33 bp, synthetic construct
  misc_feature 1..33: note = teR6-H5A(T-1N)-R2
  source 1..33: mol_type = other DNA
cgaagcttaacacggaatataatttgcattacc

SEQ ID NO: 153 - DNA, 33 bp, synthetic construct
  misc_feature 1..33: note = teR6-H5A(T-1P)-R2
  source 1..33: mol_type = other DNA
cgaagcttaacacggaatatacggtgcattacc

SEQ ID NO: 154 - DNA, 33 bp, synthetic construct
  misc_feature 1..33: note = teR6-H5A(T-1Q)-R2
  source 1..33: mol_type = other DNA
cgaagcttaacacggaatatattgtgcattacc

SEQ ID NO: 155 - DNA, 33 bp, synthetic construct
  misc_feature 1..33: note = teR6-H5A(T-1R)-R2
  source 1..33: mol_type = other DNA
cgaagcttaacacggaatataacgtgcattacc

SEQ ID NO: 156 - DNA, 33 bp, synthetic construct
  misc_feature 1..33: note = teR6-H5A(T-1S)-R2
  source 1..33: mol_type = other DNA
cgaagcttaacacggaatataagatgcattacc

SEQ ID NO: 157 - DNA, 33 bp, synthetic construct
  misc_feature 1..33: note = teR6-H5A(T-1V)-R2
  source 1..33: mol_type = other DNA
cgaagcttaacacggaatataaactgcattacc

SEQ ID NO: 158 - DNA, 33 bp, synthetic construct
  misc_feature 1..33: note = teR6-H5A(T-1W)-R2
  source 1..33: mol_type = other DNA
cgaagcttaacacggaatataccatgcattacc

SEQ ID NO: 159 - DNA, 33 bp, synthetic construct
  misc_feature 1..33: note = teR6-H5A(T-1Y)-R2
  source 1..33: mol_type = other DNA
cgaagcttaacacggaatataatatgcattacc

SEQ ID NO: 160 - DNA, 35 bp, synthetic construct
  misc_feature 1..35: note = Lim-E54A-Forward
  source 1..35: mol_type = other DNA
cattattgcgtgttcaggcaagatcaaacaagacc

SEQ ID NO: 161 - DNA, 33 bp, synthetic construct
  misc_feature 1..33: note = Lim-E54A-Reverse
  source 1..33: mol_type = other DNA
gaacacgcaataatgcaatctccggtagttgcg

SEQ ID NO: 162 - DNA, 35 bp, synthetic construct
  misc_feature 1..35: note = Lim-E54Q-Forward
  source 1..35: mol_type = other DNA
cattattcagtgttcaggcaagatcaaacaagacc

SEQ ID NO: 163 - DNA, 33 bp, synthetic construct
  misc_feature 1..33: note = Lim-E54Q-Reverse
  source 1..33: mol_type = other DNA
gaacactgaataatgcaatctccggtagttgcg

SEQ ID NO: 164 - DNA, 26 bp, synthetic construct
  misc_feature 1..26: note = Lim-D70A-Forward
  source 1..26: mol_type = other DNA
cgcatccttctgcagtttagcgataa

SEQ ID NO: 165 - DNA, 27 bp, synthetic construct
  misc_feature 1..27: note = Lim-D70A-Reverse
  source 1..27: mol_type = other DNA
ctgcagaaggatgcgcgcaggatacag

SEQ ID NO: 166 - DNA, 32 bp, synthetic construct
  misc_feature 1..32: note = Lim-H172L-Forward
  source 1..32: mol_type = other DNA
taccttactgatcggctttgacttctacctcg

SEQ ID NO: 167 - DNA, 31 bp, synthetic construct
  misc_feature 1..31: note = Lim-H172L-Reverse
  source 1..31: mol_type = other DNA
ccgatcagtaaggtatcagagcgcagcatgg

SEQ ID NO: 168 - DNA, 32 bp, synthetic construct
  misc_feature 1..32: note = Lim-H172F-Forward
  source 1..32: mol_type = other DNA
taccttatttatcggctttgacttctacctcg

SEQ ID NO: 169 - DNA, 31 bp, synthetic construct
  misc_feature 1..31: note = Lim-H172F-Reverse
  source 1..31: mol_type = other DNA
ccgataaataaggtatcagagcgcagcatgg

SEQ ID NO: 170 - DNA, 32 bp, synthetic construct
  misc_feature 1..32: note = Lim-H172A-Forward
  source 1..32: mol_type = other DNA
taccttagcgatcggctttgacttctacctcg

SEQ ID NO: 171 - DNA, 31 bp, synthetic construct
  misc_feature 1..31: note = Lim-H172A-Reverse
  source 1..31: mol_type = other DNA
ccgatcgctaaggtatcagagcgcagcatgg

SEQ ID NO: 172 - protein, 63 aa, Limnothrix sp. CACIAM 69d
MPLTQLEAKTMKKDLKALMPQTVAPVQRETSATVSRDGNAITPHKYSLQGFGVMIPFAGDDAE

SEQ ID NO: 173 - protein, 31 aa, Limnothrix sp. CACIAM 69d
ETSATVSRDGNAITPHRYPHEEIPFAGDDAE

SEQ ID NO: 174 - protein, 59 aa, Limnothrix sp. CACIAM 69d
MPLTQLEAKTMKKDLKALMPQTVAPVQRETSATVSRDGNAITPHITNIFYDPFAGDDAE

SEQ ID NO: 175 - protein, 40 aa, Microcystis aeruginosa PCC 7005
RNDAPVQREINTTSSEGGTGLTPSMSGVDYYNPFAGDDAE

SEQ ID NO: 176 - protein, 48 aa, Planktothrix agardhii
MTKKNLKPQQAAPVQREINTTSSESGTSTGLTPHINPYLYPFAGDDAE

SEQ ID NO: 177 - protein, 47 aa, Anabaena sp. UHCC-0232
MTKKNIRPQQVAPVQRETISNAKDQSGQVTPHHQPWHAAPFAGDDAE

SEQ ID NO: 178 - protein, 12 aa, Limnothrix sp. CACIAM 69d
KYSLQGFGVMIP

SEQ ID NO: 179 - protein, 8 aa, Limnothrix sp. CACIAM 69d
RYPHEEIP

SEQ ID NO: 180 - protein, 8 aa, Limnothrix sp. CACIAM 69d
ITNIFYDP

SEQ ID NO: 181 - protein, 8 aa, Limnothrix sp. CACIAM 69d
  SITE 4: note = X is geranylated histidine
RYPXEEIP

SEQ ID NO: 182 - DNA, 33 bp, synthetic construct
  misc_feature 1..33: note = DNA encording teLimE2
  source 1..33: mol_type = other DNA
atgcgttatccgcatgaagaaattccgtgttaa

SEQ ID NO: 183 - protein, 7 aa, unidentified
  REGION 1..7: note = Substrate for PagF
INPYLYP

SEQ ID NO: 184 - protein, 10 aa, unidentified
  REGION 1..10: note = Substrate for AcyF
TSQIWGSPVP

SEQ ID NO: 185 - protein, 7 aa, unidentified
  REGION 1..7: note = Substrate for LynF
APMPPYP

SEQ ID NO: 186 - protein, 9 aa, unidentified
  REGION 1..9: note = Substrate for PirF
MSGVDYYNP

SEQ ID NO: 187 - protein, 16 aa, unidentified
  REGION 1..16: note = Substrate for PirF
MSGVDYYNPFAGDDAE

SEQ ID NO: 188 - protein, 32 aa, synthetic construct
  REGION 1..32: note = long linear substrate for LimF
METSATVSRDGNAITPHRYPHEEIPFAGDDAE

SEQ ID NO: 189 - protein, 16 aa, synthetic construct
  REGION 1..16: note = middle linear substrate for LimF
MRYPHEEIPFAGDDAE

SEQ ID NO: 190 - protein, 9 aa, synthetic construct
  REGION 1..9: note = short linear substrate for LimF
MRYPHEEIP

SEQ ID NO: 191 - protein, 31 aa, synthetic construct
  REGION 1..31: note = Elcatonin
  SITE 6: note = X is alpha-aminosuberic acid
SNLSTXVLGKLSQELHKLQTYPRTDVGAGTP

SEQ ID NO: 192 - protein, 8 aa, Homo sapiens
DRVYIHPF

SEQ ID NO: 193 - protein, 10 aa, Homo sapiens
  SITE 1: note = X is pyroglutamic acid
XHWSYGLRPG

SEQ ID NO: 194 - protein, 13 aa, Saccharomyces cerevisiae
WHWLQLKPGQPMY

SEQ ID NO: 195 - protein, 28 aa, synthetic construct
  REGION 1..28: note = Aviptadil
HSDAVFTDNYTRLRKQMAVKKYLNSILN

SEQ ID NO: 196 - protein, 37 aa, synthetic construct
  REGION 1..37: note = Pramlintide
KCNTATCATQRLANFLVHSSNNFGPILPPTNVGSNTY

SEQ ID NO: 197 - protein, 30 aa, Homo sapiens
HAEGTFTSDVSSYLEGQAAKEFIAWLVKGR

SEQ ID NO: 198 - protein, 33 aa, synthetic construct
  REGION 1..33: note = Teduglutide
HGDGSFSDEMNTILDNLAARDFINWLIQTKITD

SEQ ID NO: 199 - protein, 15 aa, Homo sapiens
PGTCEICAYAACTGC

SEQ ID NO: 200 - protein, 13 aa, Saccharomyces cerevisiae
WHWLQLKPGQPMY

SEQ ID NO: 201 - protein, 5 aa, Homo sapiens
YGGFL

SEQ ID NO: 202 - protein, 8 aa, Homo sapiens
DRVYIHPF

SEQ ID NO: 203 - protein, 17 aa, Homo sapiens
  SITE 1: note = X is pyroglutamic acid
XGPWLEEEEEAYGWMDF

SEQ ID NO: 204 - protein, 30 aa, synthetic construct
FAEGTFTSDVSSYLEGQAAKEFIAWLVHGR